European Patent Specification EP 3 853 360 B1, published July 15, 2026. Title: Trypsin mutant for C- and N-terminal modification of polypeptides. Applicant: BIOPHARMA TRANSLATIONSINSTITUT DESSAU FORSCHUNGS GMBH. The sequence listing filed with the application follows.

SEQUENCE LISTING (60 sequences)

SEQ ID NO: 1 - protein, 223 aa, Rattus norvegicus
  mature anionic rat trypsin II
IVGGYTCQENSVPYQVSLNSGYHFCGGSLINDQWVVSAAHCYKSRIQVRLGEHNINVLEGNEQFVNAAKIIKHPNFDRKTLNNDIMLIKLSSPVKLNARVATVALPSSCAPAGTQCLISGWGNTLSSGVNEPDLLQCLDAPLLPQADCEASYPGKITDNMVCVGFLEGGKDSCQGDSGGPVVCNGELQGIVSWGYGCALPDNPGVYTKVCNYVDWIQDTIAAN

SEQ ID NO: 2 - protein, 245 aa, Artificial Sequence
  anti-Her2-Fab-YRAH heavy chain
EVKLQESGGGLVQPGGSLRLSCAASGFNIKDTYIHWVRQAPGKGLEWVARIYPTNGYTRYADSVKGRFTISADTSKNTAYLQMNSLRAEDTAVYYCSRWGGDGFYAMDYWGQGTLVTVSSASTKGPSVFPLAPSSKSTSGGTAALGCLVKDYFPEPVTVSWNSGALTSGVHTFPAVLQSSGLYSLSSVVTVPSSSLGTQTYICNVNHKPSNTKVDKKVEPKSCADKPGGYRAHAGEQKLISEEDL

SEQ ID NO: 3 - protein, 214 aa, Artificial Sequence
  anti-Her2-Fab-YRAH light chain
DIELTQSPSSLSASVGDRVTITCRASQDVNTAVAWYQQKPGKAPKLLIYSASFLYSGVPSRFSGSRSGTDFTLTISSLQPEDFATYYCQQHYTTPPTFGQGTKLEIKRTVAAPSVFIFPPSDEQLKSGTASVVCLLNNFYPREAKVQWKVDNALQSGNSQESVTEQDSKDSTYSLSSTLTLSKADYEKHKVYACEVTHQGLSSPVTKSFNRGEC

SEQ ID NO: 4 - protein, 184 aa, Artificial Sequence
  Strep-YRAH-cyclophilin18
GWSHPQFEKYRAHAVNPTVFFDIAVDGEPLGRVSFELFADKVPKTAENFRALSTGEKGFGYKGSCFHRIIPGFMCQGGDFTRHNGTGGKSIYGEKFEDENFILKHTGPGILSMANAGPNTNGSQFFICTAKTEWLDGKHVVFGKVKEGMNIVEAMERFGSRNGKTSKKITIADCGQLAYRHAAG

SEQ ID NO: 5 - protein, 449 aa, Artificial Sequence
  anti-Her2-antibody RAH-Trastuzumab heavy chain
EVQLVESGGGLVQPGGSLRLSCAASGFNIKDTYIHWVRQAPGKGLEWVARIYPTNGYTRYADSVKGRFTISADTSKNTAYLQMNSLRAEDTAVYYCSRWGGDGFYAMDYWGQGTLVTVSSASTKGPSVFPLAPSSKSTSGGTAALGCLVKDYFPEPVTVSWNSGALTSGVHTFPAVLQSSGLYSLSSVVTVPSSSLGTQTYICNVNHKPSNTKVDKKVEPKSCDKTHTCPPCPAPELLGGPSVFLFPPKPKDTLMISRTPEVTCVVVDVSHEDPEVKFNWYVDGVEVHNAKTKPREEQYNSTYRVVSVLTVLHQDWLNGKEYKCKVSNKALPAPIEKTISKAKGQPREPQVYTLPPSREEMTKNQVSLTCLVKGFYPSDIAVEWESNGQPENNYKTTPPVLDSDGSFFLYSKLTVDKSRWQQGNVFSCSVMHEALHNHYTQKSLSLSPG

SEQ ID NO: 6 - protein, 218 aa, Artificial Sequence
  anti-Her2-antibody RAH-Trastuzumab light chain
RAHADIQMTQSPSSLSASVGDRVTITCRASQDVNTAVAWYQQKPGKAPKLLIYSASFLYSGVPSRFSGSRSGTDFTLTISSLQPEDFATYYCQQHYTTPPTFGQGTKVEIKRTVAAPSVFIFPPSDEQLKSGTASVVCLLNNFYPREAKVQWKVDNALQSGNSQESVTEQDSKDSTYSLSSTLTLSKADYEKHKVYACEVTHQGLSSPVTKSFNRGEC

SEQ ID NO: 7 - protein, 5 aa, Artificial Sequence
  polypeptide
YRAAG

SEQ ID NO: 8 - protein, 6 aa, Artificial Sequence
  polypeptide
YRHAAG

SEQ ID NO: 9 - protein, 7 aa, Artificial Sequence
  polypeptide
YRAHAAG

SEQ ID NO: 10 - protein, 9 aa, Artificial Sequence
  polypeptide
AAYRAAHAG

SEQ ID NO: 11 - protein, 9 aa, Artificial Sequence
  polypeptide
AAYRAHAAG

SEQ ID NO: 12 - protein, 9 aa, Artificial Sequence
  polypeptide
AAYRHAAAG

SEQ ID NO: 13 - protein, 4 aa, Artificial Sequence
  polypeptide
AHAG

SEQ ID NO: 14 - protein, 5 aa, Artificial Sequence
  polypeptide
AAHAG

SEQ ID NO: 15 - protein, 5 aa, Artificial Sequence
  polypeptide
RAHAK

SEQ ID NO: 16 - protein, 5 aa, Artificial Sequence
  polypeptide
RAAHK

SEQ ID NO: 17 - protein, 4 aa, Artificial Sequence
  polypeptide
RHAK

SEQ ID NO: 18 - protein, 5 aa, Artificial Sequence
  polypeptide
RAHAK

SEQ ID NO: 19 - protein, 9 aa, Artificial Sequence
  polypeptide
PGGYRKDAG

SEQ ID NO: 20 - protein, 9 aa, Artificial Sequence
  polypeptide
PGGYRKKAG

SEQ ID NO: 21 - protein, 9 aa, Artificial Sequence
  polypeptide
PGGYRKNAG

SEQ ID NO: 22 - protein, 9 aa, Artificial Sequence
  polypeptide
PGGYRKAAG

SEQ ID NO: 23 - protein, 9 aa, Artificial Sequence
  polypeptide
PGGYRRHAG

SEQ ID NO: 24 - protein, 9 aa, Artificial Sequence
  Artificial Sequence
PGGYDKHAG

SEQ ID NO: 25 - protein, 9 aa, Artificial Sequence
  polypeptide
PGGYAKHAG

SEQ ID NO: 26 - protein, 9 aa, Artificial Sequence
  polypeptide
PGGARKHAG

SEQ ID NO: 27 - protein, 9 aa, Artificial Sequence
  polypeptide
PGGDRKHAG

SEQ ID NO: 28 - protein, 9 aa, Artificial Sequence
  polypeptide
PGGRRKHAG

SEQ ID NO: 29 - protein, 9 aa, Artificial Sequence
  polypeptide
PGGLRKHAG

SEQ ID NO: 30 - protein, 9 aa, Artificial Sequence
  polypeptide
PGGWRKHAG

SEQ ID NO: 31 - protein, 9 aa, Artificial Sequence
  polypeptide
PGGFRKHAG

SEQ ID NO: 32 - protein, 9 aa, Artificial Sequence
  polypeptide
PGGYRKHAG

SEQ ID NO: 33 - protein, 9 aa, Artificial Sequence
  polypeptide
PGGYRADAG

SEQ ID NO: 34 - protein, 9 aa, Artificial Sequence
  polypeptide
PGGYRAKAG

SEQ ID NO: 35 - protein, 9 aa, Artificial Sequence
  polypeptide
PGGYRANAG

SEQ ID NO: 36 - protein, 9 aa, Artificial Sequence
  polypeptide
PGGYRAAAG

SEQ ID NO: 37 - protein, 9 aa, Artificial Sequence
  polypeptide
PGGYKAHAG

SEQ ID NO: 38 - protein, 9 aa, Artificial Sequence
  Artificial Sequence
PGGYDAHAG

SEQ ID NO: 39 - protein, 9 aa, Artificial Sequence
  polypeptide
PGGYAAHAG

SEQ ID NO: 40 - protein, 9 aa, Artificial Sequence
  polypeptide
PGGARAHAG

SEQ ID NO: 41 - protein, 9 aa, Artificial Sequence
  polypeptide
PGGDRAHAG

SEQ ID NO: 42 - protein, 9 aa, Artificial Sequence
  polypeptide
PGGRRAHAG

SEQ ID NO: 43 - protein, 9 aa, Artificial Sequence
  polypeptide
PGGWRAHAG

SEQ ID NO: 44 - protein, 9 aa, Artificial Sequence
  polypeptide
PGGFRAHAG

SEQ ID NO: 45 - protein, 9 aa, Artificial Sequence
  polypeptide
PGGYRAHAG

SEQ ID NO: 46 - protein, 5 aa, Artificial Sequence
  polypeptide
RKDAK

SEQ ID NO: 47 - protein, 5 aa, Artificial Sequence
  polypeptide
RKKAK

SEQ ID NO: 48 - protein, 6 aa, Artificial Sequence
  polypeptide
BRKNAK

SEQ ID NO: 49 - protein, 5 aa, Artificial Sequence
  polypeptide
RKAAK

SEQ ID NO: 50 - protein, 5 aa, Artificial Sequence
  polypeptide
RRHAK

SEQ ID NO: 51 - protein, 5 aa, Artificial Sequence
  polypeptide
DKHAK

SEQ ID NO: 52 - protein, 5 aa, Artificial Sequence
  polypeptide
AKHAK

SEQ ID NO: 53 - protein, 5 aa, Artificial Sequence
  polypeptide
RKHAK

SEQ ID NO: 54 - protein, 5 aa, Artificial Sequence
  polypeptide
RADAK

SEQ ID NO: 55 - protein, 5 aa, Artificial Sequence
  polypeptide
RAKAK

SEQ ID NO: 56 - protein, 5 aa, Artificial Sequence
  polypeptide
RANAK

SEQ ID NO: 57 - protein, 5 aa, Artificial Sequence
  polypeptide
RAAAK

SEQ ID NO: 58 - protein, 5 aa, Artificial Sequence
  polypeptide
KAHAK

SEQ ID NO: 59 - protein, 5 aa, Artificial Sequence
  polypeptide
DAHAK

SEQ ID NO: 60 - protein, 5 aa, Artificial Sequence
  polypeptide
AAHAK